European Patent Application EP 4 624 577 A1, published October 1, 2025. Title: Multifunctional system. Applicant: Ospedale San Raffaele S.r.l. The sequence listing filed with the application follows.

SEQUENCE LISTING (9 sequences)

SEQ ID NO: 1 - RNA, 34 nt, synthetic construct
  source 1..34: mol_type = other RNA
gcggacggacagagagtgcaacctgccgtgccgc

SEQ ID NO: 2 - RNA, 34 nt, synthetic construct; identical to SEQ ID NO: 1
  source 1..34: mol_type = other RNA
  modified_base 2: mod_base = OTHER; note = 2'-fluorocytidine
  modified_base 6: mod_base = OTHER; note = 2'-fluorocytidine
  modified_base 10: mod_base = OTHER; note = 2'-fluorocytidine
  modified_base 17: mod_base = OTHER; note = 2'-fluorouridine
  modified_base 19: mod_base = OTHER; note = 2'-fluorocytidine
  modified_base 22: mod_base = OTHER; note = 2'-fluorocytidine
  modified_base 23: mod_base = OTHER; note = 2'-fluorocytidine
  modified_base 24: mod_base = OTHER; note = 2'-fluorouridine
  modified_base 26: mod_base = OTHER; note = 2'-fluorocytidine
  modified_base 27: mod_base = OTHER; note = 2'-fluorocytidine
  modified_base 29: mod_base = OTHER; note = 2'-fluorouridine
  modified_base 31: mod_base = OTHER; note = 2'-fluorocytidine
  modified_base 32: mod_base = OTHER; note = 2'-fluorocytidine
  modified_base 34: mod_base = OTHER; note = 2'-fluorocytidine

SEQ ID NO: 3 - DNA, 15 bp, synthetic construct
  source 1..15: mol_type = other DNA
agcggacggacagag

SEQ ID NO: 4 - DNA, 15 bp, synthetic construct
  source 1..15: mol_type = other DNA
gcggcacggcaggtt

SEQ ID NO: 5 - DNA, 32 bp, synthetic construct
  source 1..32: mol_type = other DNA
taatacgactcactatagggttcgtaccgggt

SEQ ID NO: 6 - DNA, 18 bp, synthetic construct
  source 1..18: mol_type = other DNA
tgacacgttctatgtgca

SEQ ID NO: 7 - RNA, 34 nt, synthetic construct; identical to SEQ ID NO: 1
  source 1..34: mol_type = other RNA
  modified_base 1: mod_base = OTHER; note = modified with C6-thiol
  modified_base 2: mod_base = OTHER; note = 2'-fluorocytidine
  modified_base 6: mod_base = OTHER; note = 2'-fluorocytidine
  modified_base 10: mod_base = OTHER; note = 2'-fluorocytidine
  modified_base 17: mod_base = OTHER; note = 2'-fluorouridine
  modified_base 19: mod_base = OTHER; note = 2'-fluorocytidine
  modified_base 22: mod_base = OTHER; note = 2'-fluorocytidine
  modified_base 23: mod_base = OTHER; note = 2'-fluorocytidine
  modified_base 24: mod_base = OTHER; note = 2'-fluorouridine
  modified_base 26: mod_base = OTHER; note = 2'-fluorocytidine
  modified_base 27: mod_base = OTHER; note = 2'-fluorocytidine
  modified_base 29: mod_base = OTHER; note = 2'-fluorouridine
  modified_base 31: mod_base = OTHER; note = 2'-fluorocytidine
  modified_base 32: mod_base = OTHER; note = 2'-fluorocytidine
  modified_base 34: mod_base = OTHER; note = 2'-fluorocytidine

SEQ ID NO: 8 - RNA, 39 nt, synthetic construct
  source 1..39: mol_type = other RNA
  modified_base 1: mod_base = OTHER; note = 2'-fluorouridine
  modified_base 2: mod_base = OTHER; note = 2'-fluorouridine
  modified_base 3: mod_base = OTHER; note = 2'-fluorocytidine
  modified_base 5: mod_base = OTHER; note = 2'-fluorouridine
  modified_base 7: mod_base = OTHER; note = 2'-fluorocytidine
  modified_base 8: mod_base = OTHER; note = 2'-fluorocytidine
  modified_base 12: mod_base = OTHER; note = 2'-fluorouridine
  modified_base 16: mod_base = OTHER; note = 2'-fluorouridine
  modified_base 20: mod_base = OTHER; note = 2'-fluorocytidine
  modified_base 21: mod_base = OTHER; note = 2'-fluorouridine
  modified_base 22: mod_base = OTHER; note = 2'-fluorouridine
  modified_base 24: mod_base = OTHER; note = 2'-fluorocytidine
  modified_base 26: mod_base = OTHER; note = 2'-fluorocytidine
  modified_base 28: mod_base = OTHER; note = 2'-fluorouridine
  modified_base 33: mod_base = OTHER; note = 2'-fluorocytidine
  modified_base 35: mod_base = OTHER; note = 2'-fluorouridine
  modified_base 37: mod_base = OTHER; note = 2'-fluorouridine
  modified_base 38: mod_base = OTHER; note = 2'-fluorocytidine
  modified_base 17: mod_base = OTHER; note = 2'-fluorouridine
ttcgtaccgggtaggttggcttgcacatagaacgtgtca

SEQ ID NO: 9 - RNA, 39 nt, synthetic construct; identical to SEQ ID NO: 8
  source 1..39: mol_type = other RNA
  modified_base 1: mod_base = OTHER; note = 2'-fluorouridine
  modified_base 2: mod_base = OTHER; note = 2'-fluorouridine
  modified_base 3: mod_base = OTHER; note = 2'-fluorocytidine
  modified_base 5: mod_base = OTHER; note = 2'-fluorouridine
  modified_base 7: mod_base = OTHER; note = 2'fluorocytidine
  modified_base 8: mod_base = OTHER; note = 2'-fluorocytidine
  modified_base 12: mod_base = OTHER; note = 2'-fluorouridine
  modified_base 16: mod_base = OTHER; note = 2'-fluorouridine
  modified_base 20: mod_base = OTHER; note = 2'-fluorocytidine
  modified_base 21: mod_base = OTHER; note = 2'-fluorouridine
  modified_base 22: mod_base = OTHER; note = 2'-fluorouridine
  modified_base 24: mod_base = OTHER; note = 2'-fluorocytidine
  modified_base 26: mod_base = OTHER; note = 2'-fluorocytidine
  modified_base 28: mod_base = OTHER; note = 2'-fluorouridine
  modified_base 33: mod_base = OTHER; note = 2'-fluorocytidine
  modified_base 35: mod_base = OTHER; note = 2'-fluorouridine
  modified_base 37: mod_base = OTHER; note = 2'-fluorouridine
  modified_base 38: mod_base = OTHER; note = 2'-fluorocytidine
  modified_base 1: mod_base = OTHER; note = modified at 5' with C6-thiol
  modified_base 17: mod_base = OTHER; note = 2'-fluorouridine